European Patent Application EP 4 417 627 A1, published August 21, 2024. Title: 重组融合抗体和抗体-药物偶联物及其用途. Applicant: 中山大学. The sequence listing filed with the application follows.

SEQUENCE LISTING (66 sequences)

SEQ ID NO: 1 - protein, 13 aa, synthetic construct
ASVSLLDDELMSL

SEQ ID NO: 2 - protein, 16 aa, synthetic construct
RRRASVSLLDDELMSL

SEQ ID NO: 3 - protein, 10 aa, synthetic construct
ASVSLLDDEL

SEQ ID NO: 4 - protein, 13 aa, synthetic construct
ASSGLDDLDLLGK

SEQ ID NO: 5 - protein, 13 aa, synthetic construct
VQNPSADRNLLDL

SEQ ID NO: 6 - protein, 13 aa, synthetic construct
NALSWLDEELLCL

SEQ ID NO: 7 - protein, 8 aa, synthetic construct
SDEDLLHI

SEQ ID NO: 8 - protein, 13 aa, synthetic construct
SFHDDSDEDLLHI

SEQ ID NO: 9 - protein, 13 aa, synthetic construct
EESEERDDHLLPM

SEQ ID NO: 10 - protein, 10 aa, synthetic construct
SYKYSKVNKE

SEQ ID NO: 11 - protein, 10 aa, synthetic construct
PAAYRGVGDD

SEQ ID NO: 12 - protein, 11 aa, synthetic construct
RRRSDEDLLHI

SEQ ID NO: 13 - protein, 13 aa, synthetic construct
RRLRKSDEDLLHI

SEQ ID NO: 14 - protein, 13 aa, synthetic construct
RRRRKSDEDLLHI

SEQ ID NO: 15 - protein, 16 aa, synthetic construct
RRRSFHDDSDEDLLHI

SEQ ID NO: 16 - protein, 18 aa, synthetic construct
RRLRKSFHDDSDEDLLHI

SEQ ID NO: 17 - protein, 18 aa, synthetic construct
RRRRKSFHDDSDEDLLHI

SEQ ID NO: 18 - protein, 11 aa, synthetic construct
RKRSHAGYQTI

SEQ ID NO: 19 - protein, 16 aa, synthetic construct
RRRRKRKRSHAGYQTI

SEQ ID NO: 20 - protein, 10 aa, synthetic construct
KHHHAGYEQF

SEQ ID NO: 21 - protein, 14 aa, synthetic construct
RRLRKHHHAGYEQF

SEQ ID NO: 22 - protein, 7 aa, synthetic construct
LPETGGG

SEQ ID NO: 23 - protein, 5 aa, synthetic construct
GGGGG

SEQ ID NO: 24 - protein, 5 aa, synthetic construct
GGGGS

SEQ ID NO: 25 - protein, 10 aa, synthetic construct
GGGGSGGGGS

SEQ ID NO: 26 - protein, 15 aa, synthetic construct
GGGGSGGGGSGGGGS

SEQ ID NO: 27 - protein, 118 aa, synthetic construct
EVQLVESGGGLVQAGGSLRLSCAASGITFSINTMGWYRQAPGKQRELVALISSIGDTYYADSVKGRFTISRDNAKNTVYLQMNSLKPEDTAVYYCKRFRTAAQGTDYWGQGTQVTVSS

SEQ ID NO: 28 - protein, 118 aa, synthetic construct
EVQLVESGGGLVQAGGSLRLSCAASGITFSINTMGWYRQAPGKQRELVALISSIGDTYYADSVKGRFTISRDNAKNTVYLQMNCLKPEDTAVYYCKRFRTAAQGTDYWGQGTQVTVSS

SEQ ID NO: 29 - protein, 450 aa, synthetic construct
EVQLVESGGGLVQPGGSLRLSCAASGFNIKDTYIHWVRQAPGKGLEWVARIYPTNGYTRYADSVKGRFTISADTSKNTAYLQMNSLRAEDTAVYYCSRWGGDGFYAMDYWGQGTLVTVSSASTKGPSVFPLAPSSKSTSGGTAALGCLVKDYFPEPVTVSWNSGALTSGVHTFPAVLQSSGLYSLSSVVTVPSSSLGTQTYICNVNHKPSNTKVDKKVEPKSCDKTHTCPPCPAPELLGGPSVFLFPPKPKDTLMISRTPEVTCVVVDVSHEDPEVKFNWYVDGVEVHNAKTKPREEQYNSTYRVVSVLTVLHQDWLNGKEYKCKVSNKALPAPIEKTISKAKGQPREPQVYTLPPSREEMTKNQVSLTCLVKGFYPSDIAVEWESNGQPENNYKTTPPVLDSDGSFFLYSKLTVDKSRWQQGNVFSCSVMHEALHNHYTQKSLSLSPGK

SEQ ID NO: 30 - protein, 450 aa, synthetic construct
EVQLVESGGGLVQPGGSLRLSCAASGFNIKDTYIHWVRQAPGKGLEWVARIYPTNGYTRYADSVKGRFTISADTSKNTAYLQMNSLRAEDTAVYYCSRWGGDGFYAMDYWGQGTLVTVSSCSTKGPSVFPLAPSSKSTSGGTAALGCLVKDYFPEPVTVSWNSGALTSGVHTFPAVLQSSGLYSLSSVVTVPSSSLGTQTYICNVNHKPSNTKVDKKVEPKSCDKTHTCPPCPAPELLGGPSVFLFPPKPKDTLMISRTPEVTCVVVDVSHEDPEVKFNWYVDGVEVHNAKTKPREEQYNSTYRVVSVLTVLHQDWLNGKEYKCKVSNKALPAPIEKTISKAKGQPREPQVYTLPPSREEMTKNQVSLTCLVKGFYPSDIAVEWESNGQPENNYKTTPPVLDSDGSFFLYSKLTVDKSRWQQGNVFSCSVMHEALHNHYTQKSLSLSPGK

SEQ ID NO: 31 - protein, 214 aa, synthetic construct
DIQMTQSPSSLSASVGDRVTITCRASQDVNTAVAWYQQKPGKAPKLLIYSASFLYSGVPSRFSGSRSGTDFTLTISSLQPEDFATYYCQQHYTTPPTFGQGTKVEIKRTVAAPSVFIFPPSDEQLKSGTASVVCLLNNFYPREAKVQWKVDNALQSGNSQESVTEQDSKDSTYSLSSTLTLSKADYEKHKVYACEVTHQGLSSPVTKSFNRGEC

SEQ ID NO: 32 - protein, 124 aa, synthetic construct
EVQLVESGGGLVQAGGSLRLSCAASGITFSINTMGWYRQAPGKQRELVALISSIGDTYYADSVKGRFTISRDNAKNTVYLQMNCLKPEDTAVYYCKRFRTAAQGTDYWGQGTQVTVSSHHHHHH

SEQ ID NO: 33 - protein, 144 aa, synthetic construct
EVQLVESGGGLVQAGGSLRLSCAASGITFSINTMGWYRQAPGKQRELVALISSIGDTYYADSVKGRFTISRDNAKNTVYLQMNCLKPEDTAVYYCKRFRTAAQGTDYWGQGTQVTVSSHHHHHHLPETGGGASVSLLDDELMSL

SEQ ID NO: 34 - protein, 147 aa, synthetic construct
EVQLVESGGGLVQAGGSLRLSCAASGITFSINTMGWYRQAPGKQRELVALISSIGDTYYADSVKGRFTISRDNAKNTVYLQMNCLKPEDTAVYYCKRFRTAAQGTDYWGQGTQVTVSSHHHHHHLPETGGGRRRASVSLLDDELMSL

SEQ ID NO: 35 - protein, 141 aa, synthetic construct
EVQLVESGGGLVQAGGSLRLSCAASGITFSINTMGWYRQAPGKQRELVALISSIGDTYYADSVKGRFTISRDNAKNTVYLQMNCLKPEDTAVYYCKRFRTAAQGTDYWGQGTQVTVSSHHHHHHLPETGGGASVSLLDDEL

SEQ ID NO: 36 - protein, 145 aa, synthetic construct
EVQLVESGGGLVQAGGSLRLSCAASGITFSINTMGWYRQAPGKQRELVALISSIGDTYYADSVKGRFTISRDNAKNTVYLQMNCLKPEDTAVYYCKRFRTAAQGTDYWGQGTQVTVSSHHHHHHHLPETGGGASSGLDDLDLLGK

SEQ ID NO: 37 - protein, 144 aa, synthetic construct
EVQLVESGGGLVQAGGSLRLSCAASGITFSINTMGWYRQAPGKQRELVALISSIGDTYYADSVKGRFTISRDNAKNTVYLQMNCLKPEDTAVYYCKRFRTAAQGTDYWGQGTQVTVSSHHHHHHLPETGGGVQNPSADRNLLDL

SEQ ID NO: 38 - protein, 145 aa, synthetic construct
EVQLVESGGGLVQAGGSLRLSCAASGITFSINTMGWYRQAPGKQRELVALISSIGDTYYADSVKGRFTISRDNAKNTVYLQMNCLKPEDTAVYYCKRFRTAAQGTDYWGQGTQVTVSSHHHHHHHLPETGGGNALSWLDEELLCL

SEQ ID NO: 39 - protein, 139 aa, synthetic construct
EVQLVESGGGLVQAGGSLRLSCAASGITFSINTMGWYRQAPGKQRELVALISSIGDTYYADSVKGRFTISRDNAKNTVYLQMNCLKPEDTAVYYCKRFRTAAQGTDYWGQGTQVTVSSHHHHHHLPETGGGSDEDLLHI

SEQ ID NO: 40 - protein, 139 aa, synthetic construct
EVQLVESGGGLVQAGGSLRLSCAASGITFSINTMGWYRQAPGKQRELVALISSIGDTYYADSVKGRFTISRDNAKNTVYLQMNCLKPEDTAVYYCKRFRTAAQGTDYWGQGTQVTVSSLPETGGGSDEDLLHIHHHHHH

SEQ ID NO: 41 - protein, 135 aa, synthetic construct
EVQLVESGGGLVQAGGSLRLSCAASGITFSINTMGWYRQAPGKQRELVALISSIGDTYYADSVKGRFTISRDNAKNTVYLQMNCLKPEDTAVYYCKRFRTAAQGTDYWGQGTQVTVSSHHHHHHGGGSDEDLLHI

SEQ ID NO: 42 - protein, 137 aa, synthetic construct
EVQLVESGGGLVQAGGSLRLSCAASGITFSINTMGWYRQAPGKQRELVALISSIGDTYYADSVKGRFTISRDNAKNTVYLQMNCLKPEDTAVYYCKRFRTAAQGTDYWGQGTQVTVSSHHHHHHGGGGGSDEDLLHI

SEQ ID NO: 43 - protein, 137 aa, synthetic construct
EVQLVESGGGLVQAGGSLRLSCAASGITFSINTMGWYRQAPGKQRELVALISSIGDTYYADSVKGRFTISRDNAKNTVYLQMNCLKPEDTAVYYCKRFRTAAQGTDYWGQGTQVTVSSHHHHHHGGGGSSDEDLLHI

SEQ ID NO: 44 - protein, 147 aa, synthetic construct
EVQLVESGGGLVQAGGSLRLSCAASGITFSINTMGWYRQAPGKQRELVALISSIGDTYYADSVKGRFTISRDNAKNTVYLQMNCLKPEDTAVYYCKRFRTAAQGTDYWGQGTQVTVSSHHHHHHGGGGSGGGGSGGGGSSDEDLLHI

SEQ ID NO: 45 - protein, 144 aa, synthetic construct
EVQLVESGGGLVQAGGSLRLSCAASGITFSINTMGWYRQAPGKQRELVALISSIGDTYYADSVKGRFTISRDNAKNTVYLQMNCLKPEDTAVYYCKRFRTAAQGTDYWGQGTQVTVSSHHHHHHLPETGGGSFHDDSDEDLLHI

SEQ ID NO: 46 - protein, 144 aa, synthetic construct
EVQLVESGGGLVQAGGSLRLSCAASGITFSINTMGWYRQAPGKQRELVALISSIGDTYYADSVKGRFTISRDNAKNTVYLQMNCLKPEDTAVYYCKRFRTAAQGTDYWGQGTQVTVSSHHHHHHLPETGGGEESEERDDHLLPM

SEQ ID NO: 47 - protein, 141 aa, synthetic construct
EVQLVESGGGLVQAGGSLRLSCAASGITFSINTMGWYRQAPGKQRELVALISSIGDTYYADSVKGRFTISRDNAKNTVYLQMNCLKPEDTAVYYCKRFRTAAQGTDYWGQGTQVTVSSHHHHHHLPETGGGSYKYSKVNKE

SEQ ID NO: 48 - protein, 141 aa, synthetic construct
EVQLVESGGGLVQAGGSLRLSCAASGITFSINTMGWYRQAPGKQRELVALISSIGDTYYADSVKGRFTISRDNAKNTVYLQMNCLKPEDTAVYYCKRFRTAAQGTDYWGQGTQVTVSSHHHHHHLPETGGGPAAYRGVGDD

SEQ ID NO: 49 - protein, 142 aa, synthetic construct
EVQLVESGGGLVQAGGSLRLSCAASGITFSINTMGWYRQAPGKQRELVALISSIGDTYYADSVKGRFTISRDNAKNTVYLQMNCLKPEDTAVYYCKRFRTAAQGTDYWGQGTQVTVSSHHHHHHLPETGGGRRRSDEDLLHI

SEQ ID NO: 50 - protein, 143 aa, synthetic construct
EVQLVESGGGLVQAGGSLRLSCAASGITFSINTMGWYRQAPGKQRELVALISSIGDTYYADSVKGRFTISRDNAKNTVYLQMNCLKPEDTAVYYCKRFRTAAQGTDYWGQGTQVTVSSHHHHHHLPETGGGRRLRSDEDLLHI

SEQ ID NO: 51 - protein, 144 aa, synthetic construct
EVQLVESGGGLVQAGGSLRLSCAASGITFSINTMGWYRQAPGKQRELVALISSIGDTYYADSVKGRFTISRDNAKNTVYLQMNCLKPEDTAVYYCKRFRTAAQGTDYWGQGTQVTVSSHHHHHHLPETGGGRRRRKSDEDLLHI

SEQ ID NO: 52 - protein, 147 aa, synthetic construct
EVQLVESGGGLVQAGGSLRLSCAASGITFSINTMGWYRQAPGKQRELVALISSIGDTYYADSVKGRFTISRDNAKNTVYLQMNCLKPEDTAVYYCKRFRTAAQGTDYWGQGTQVTVSSHHHHHHLPETGGGRRRSFHDDSDEDLLHI

SEQ ID NO: 53 - protein, 149 aa, synthetic construct
EVQLVESGGGLVQAGGSLRLSCAASGITFSINTMGWYRQAPGKQRELVALISSIGDTYYADSVKGRFTISRDNAKNTVYLQMNCLKPEDTAVYYCKRFRTAAQGTDYWGQGTQVTVSSHHHHHHLPETGGGRRLRKSFHDDSDEDLLHI

SEQ ID NO: 54 - protein, 149 aa, synthetic construct
EVQLVESGGGLVQAGGSLRLSCAASGITFSINTMGWYRQAPGKQRELVALISSIGDTYYADSVKGRFTISRDNAKNTVYLQMNCLKPEDTAVYYCKRFRTAAQGTDYWGQGTQVTVSSHHHHHHLPETGGGRRRRKSFHDDSDEDLLHI

SEQ ID NO: 55 - protein, 143 aa, synthetic construct
EVQLVESGGGLVQAGGSLRLSCAASGITFSINTMGWYRQAPGKQRELVALISSIGDTYYADSVKGRFTISRDNAKNTVYLQMNCLKPEDTAVYYCKRFRTAAQGTDYWGQGTQVTVSSHHHHHHHLPETGGGRKRSHAGYQTI

SEQ ID NO: 56 - protein, 148 aa, synthetic construct
EVQLVESGGGLVQAGGSLRLSCAASGITFSINTMGWYRQAPGKQRELVALISSIGDTYYADSVKGRFTISRDNAKNTVYLQMNCLKPEDTAVYYCKRFRTAAQGTDYWGQGTQVTVSSHHHHHHHLPETGGGRRRRKRKRSHAGYQTI

SEQ ID NO: 57 - protein, 142 aa, synthetic construct
EVQLVESGGGLVQAGGSLRLSCAASGITFSINTMGWYRQAPGKQRELVALISSIGDTYYADSVKGRFTISRDNAKNTVYLQMNCLKPEDTAVYYCKRFRTAAQGTDYWGQGTQVTVSSHHHHHHHLPETGGGKHHHAGYEQF

SEQ ID NO: 58 - protein, 146 aa, synthetic construct
EVQLVESGGGLVQAGGSLRLSCAASGITFSINTMGWYRQAPGKQRELVALISSIGDTYYADSVKGRFTISRDNAKNTVYLQMNCLKPEDTAVYYCKRFRTAAQGTDYWGQGTQVTVSSHHHHHHHLPETGGGRRLRKHHHAGYEQF

SEQ ID NO: 59 - protein, 229 aa, synthetic construct
DIQMTQSPSSLSASVGDRVTITCRASQDVNTAVAWYQQKPGKAPKLLIYSASFLYSGVPSRFSGSRSGTDFTLTISSLQPEDFATYYCQQHYTTPPTFGQGTKVEIKRTVAAPSVFIFPPSDEQLKSGTASVVCLLNNFYPREAKVQWKVDNALQSGNSQESVTEQDSKDSTYSLSSTLTLSKADYEKHKVYACEVTHQGLSSPVTKSFNRGECLPETGGGSDEDLLHI

SEQ ID NO: 60 - protein, 465 aa, synthetic construct
EVQLVESGGGLVQPGGSLRLSCAASGFNIKDTYIHWVRQAPGKGLEWVARIYPTNGYTRYADSVKGRFTISADTSKNTAYLQMNSLRAEDTAVYYCSRWGGDGFYAMDYWGQGTLVTVSSCSTKGPSVFPLAPSSKSTSGGTAALGCLVKDYFPEPVTVSWNSGALTSGVHTFPAVLQSSGLYSLSSVVTVPSSSLGTQTYICNVNHKPSNTKVDKKVEPKSCDKTHTCPPCPAPELLGGPSVFLFPPKPKDTLMISRTPEVTCVVVDVSHEDPEVKFNWYVDGVEVHNAKTKPREEQYNSTYRVVSVLTVLHQDWLNGKEYKCKVSNKALPAPIEKTISKAKGQPREPQVYTLPPSREEMTKNQVSLTCLVKGFYPSDIAVEWESNGQPENNYKTTPPVLDSDGSFFLYSKLTVDKSRWQQGNVFSCSVMHEALHNHYTQKSLSLSPGKLPETGGGSDEDLLHI

SEQ ID NO: 61 - protein, 229 aa, synthetic construct; identical to SEQ ID NO: 59

SEQ ID NO: 62 - protein, 450 aa, synthetic construct; identical to SEQ ID NO: 30

SEQ ID NO: 63 - protein, 214 aa, synthetic construct; identical to SEQ ID NO: 31

SEQ ID NO: 64 - protein, 465 aa, synthetic construct; identical to SEQ ID NO: 60

SEQ ID NO: 65 - protein, 229 aa, synthetic construct; identical to SEQ ID NO: 59

SEQ ID NO: 66 - protein, 465 aa, synthetic construct; identical to SEQ ID NO: 60